European Patent Specification EP 3 783 031 B1, published August 2, 2023. Title: ANTIBODY AGAINST NEUROPILIN 1 AND USE THEREOF. Applicant: SAMSUNG LIFE PUBLIC WELFARE FOUNDATION. Application PCT/KR2015/013102. The sequence listing filed with the application follows.

SEQUENCE LISTING (42 sequences)

SEQ ID NO: 1 - protein, 8 aa, Artificial Sequence
  CDRH1 of 4F12
GFTFSGYA

SEQ ID NO: 2 - protein, 8 aa, Artificial Sequence
  CDRH2 of 4F12
ISPGSGST

SEQ ID NO: 3 - protein, 9 aa, Artificial Sequence
  CDRH3 of 4F12
AKRKTRFDY

SEQ ID NO: 4 - protein, 8 aa, Artificial Sequence
  CDRL1 of 4F12
SSNIGNNS

SEQ ID NO: 5 - protein, 3 aa, Artificial Sequence
  CDRL2 of 4F12
ANN

SEQ ID NO: 6 - protein, 11 aa, Artificial Sequence
  CDRL3 of 4F12
AAWDSSLNGYV

SEQ ID NO: 7 - protein, 8 aa, Artificial Sequence
  CDRH1 of 1A03 or 3H10
GFTFSSYY

SEQ ID NO: 8 - protein, 8 aa, Artificial Sequence
  CDRH2 of 1A03 or 3H10
ISPGSSNK

SEQ ID NO: 9 - protein, 9 aa, Artificial Sequence
  CDRH3 of 1A03
ARRKKSFDY

SEQ ID NO: 10 - protein, 8 aa, Artificial Sequence
  CDRL1 of 1A03 or 3H10
SSNIGNND

SEQ ID NO: 11 - protein, 3 aa, Artificial Sequence
  CDRL2 of 1A03
SDN

SEQ ID NO: 12 - protein, 11 aa, Artificial Sequence
  CDRL3 of 1A03
GAWVASLSAYV

SEQ ID NO: 13 - protein, 9 aa, Artificial Sequence
  CDRH3 of 3H10
ARRKYMFDY

SEQ ID NO: 14 - protein, 3 aa, Artificial Sequence
  CDRL2 of 3H10
SDS

SEQ ID NO: 15 - protein, 11 aa, Artificial Sequence
  CDRL3 of 3H10
ASWDSSLSGYV

SEQ ID NO: 16 - protein, 116 aa, Artificial Sequence
  VH of 4F12
EVQLLESGGGLVQPGGSLRLSCAASGFTFSGYAMSWVRQAPGKGLEWVSGISPGSGSTYYADSVKGRFTISRDNSKNTLYLQMNSLRAEDTAVYYCAKRKTRFDYWGQGTLVTVSS

SEQ ID NO: 17 - protein, 110 aa, Artificial Sequence
  VL of 4F12
QSVLTQPPSASGTPGRRVTISCSGSSSNIGNNSVYWYQQLPGTAPKLLIYANNKRPSGVPDRFSGSKSGTSASLAISGLRSEDEADYYCAAWDSSLNGYVFGGGTKLTVL

SEQ ID NO: 18 - protein, 116 aa, Artificial Sequence
  VH of 1A03
EVQLLESGGGLVQPGGSLRLSCAASGFTFSSYYMSWVRQAPGKGLEWVSAISPGSSNKYYADSVQGRFTISRDNSKNTLYLQMNSLRAEDTAVYYCARRKKSFDYWGQGTLVTVSS

SEQ ID NO: 19 - protein, 110 aa, Artificial Sequence
  VL of 1A03
QSVLTQPPSASGTPGQRVTISCSGPSSNIGNNDVSWYQQLPGTAPKLLIYSDNNRPSGVPDRFSGSKSGTSASLAISGLRSEDEADYYCGAWVASLSAYVFGGGTKLTVL

SEQ ID NO: 20 - protein, 116 aa, Artificial Sequence
  VH of 3H10
EVQLLESGGGLVQPGGSLRLSCAASGFTFSSYYMSWVRQAPGKGLEWVSAISPGSSNKYYADSVKGRFTISRDNSKNTLYLQMNSLRAEDTAVYYCARRKYMFDYWGQGTLVTVSS

SEQ ID NO: 21 - protein, 110 aa, Artificial Sequence
  VL of 3H10
QSVLTQPPSASGTPGQRVTISCTGSSSNIGNNDVYWYQQLPGTAPKLLIYSDSNRPSGVPDRFSGSKSGTSASLAISGLRSEDEADYYCASWDSSLSGYVFGGGTKLTVL

SEQ ID NO: 22 - DNA, 348 bp, Artificial Sequence
  VH of 4F12
gaggtgcagctgttggagtctgggggaggcttggtacagcctggggggtccctgagactctcctgtgcagcctctggattcacctttagcggttatgctatgagctgggtccgccaggctccagggaaggggctggagtgggtctcagggatctctcctggtagtggtagtacatattacgctgattctgtaaaaggtcggttcaccatctccagagacaattccaagaacacgctgtatctgcaaatgaacagcctgagagccgaggacacggccgtgtattactgtgcgaaacgtaagactaggttcgactactggggccagggtacactggtcaccgtgagctca

SEQ ID NO: 23 - DNA, 330 bp, Artificial Sequence
  VL of 4F12
cagtctgtgctgactcagccaccctcagcgtctgggacccccgggcggagggtcaccatctcttgtagtggctcttcatctaatattggcaataattctgtctactggtaccagcagctcccaggaacggcccccaaactcctcatctatgctaataataagcggccaagcggggtccctgaccgattctctggctccaagtctggcacctcagcctccctggccatcagtgggctccggtccgaggatgaggctgattattactgtgctgcttgggattctagcctgaatggttatgtcttcggcggaggcaccaagctgacggtccta

SEQ ID NO: 24 - DNA, 348 bp, Artificial Sequence
  VH of 1A03
gaggtgcagctgttggagtctgggggaggcttggtacagcctggggggtccctgagactctcctgtgcagcctctggattcacctttagcagttattatatgagctgggtccgccaggctccagggaaggggctggagtgggtctcagcgatctctcctggtagtagtaataaatattacgctgattctgtacaaggtcggttcaccatctccagagacaattccaagaacacgctgtatctgcaaatgaacagcctgagagccgaggacacggccgtgtattactgtgcgagaaggaagaagtcgttcgactactggggccagggtacactggtcaccgtgagctca

SEQ ID NO: 25 - DNA, 330 bp, Artificial Sequence
  VL of 1A03
cagtctgtgctgactcagccaccctcagcgtctgggacccccgggcagagggtcaccatctcttgtagtggcccttcatctaatattggcaataatgatgtctcctggtaccagcagctcccaggaacggctcccaaactcctcatctattctgataataatcggccaagcggggtccctgaccgattctctggctccaagtctggcacctcagcctccctggccatcagtgggctccggtccgaggatgaggctgattattactgtggtgcttgggttgctagcctgagtgcttatgtcttcggcggaggcaccaagctgacggtccta

SEQ ID NO: 26 - DNA, 348 bp, Artificial Sequence
  VH of 3H10
gaggtgcagctgttggagtctgggggaggcttggtacagcctggggggtccctgagactctcctgtgcagcctctggattcacctttagcagttattatatgagctgggtccgccaggctccagggaaggggctggagtgggtctcagcgatctctcctggtagtagtaataaatattacgctgattctgtaaaaggtcggttcaccatctccagagacaattccaagaacacgctgtatctgcaaatgaacagcctgagagccgaggacacggccgtgtattactgtgcgagaaggaagtatatgttcgactactggggccagggtacactggtcaccgtgagctca

SEQ ID NO: 27 - DNA, 330 bp, Artificial Sequence
  VL of 3H10
cagtctgtgctgactcagccaccctcagcgtctgggacccccgggcagagggtcaccatctcttgtactggctcttcatctaatattggcaataatgatgtctactggtaccagcagctcccaggaacggcacccaaactcctcatctattctgatagtaatcggccaagcggggtccctgaccgattctctggctccaagtctggcacctcagcctccctggccatcagtgggctccggtccgaggatgaggctgattattactgtgcttcttgggattctagcctgagtggttatgtcttcggcggaggcaccaagctgacggtccta

SEQ ID NO: 28 - protein, 25 aa, Artificial Sequence
  1A03, 3H10 & 4F12 Hv FR1
EVQLLESGGGLVQPGGSLRLSCAAS

SEQ ID NO: 29 - protein, 17 aa, Artificial Sequence
  1A03 & 3H10 Hv FR2
MSWVRQAPGKGLEWVSA

SEQ ID NO: 30 - protein, 17 aa, Artificial Sequence
  4F12 Hv FR2
MSWVRQAPGKGLEWVSG

SEQ ID NO: 31 - protein, 38 aa, Artificial Sequence
  1A03 Hv FR3
YYADSVQGRFTISRDNSKNTLYLQMNSLRAEDTAVYYC

SEQ ID NO: 32 - protein, 38 aa, Artificial Sequence
  3H10 & 4F12 Hv FR3
YYADSVKGRFTISRDNSKNTLYLQMNSLRAEDTAVYYC

SEQ ID NO: 33 - protein, 11 aa, Artificial Sequence
  1A03, 3H10 & 4F12 Hv FR4
WGQGTLVTVSS

SEQ ID NO: 34 - protein, 25 aa, Artificial Sequence
  1A03 Lv FR1
QSVLTQPPSASGTPGQRVTISCSGP

SEQ ID NO: 35 - protein, 25 aa, Artificial Sequence
  3H10 Lv FR1
QSVLTQPPSASGTPGQRVTISCTGS

SEQ ID NO: 36 - protein, 25 aa, Artificial Sequence
  4F12 Lv FR1
QSVLTQPPSASGTPGRRVTISCSGS

SEQ ID NO: 37 - protein, 17 aa, Artificial Sequence
  1A03 Lv FR2
VSWYQQLPGTAPKLLIY

SEQ ID NO: 38 - protein, 17 aa, Artificial Sequence
  3H10 Lv FR2
VYWYQQLPGTAPKLLIY

SEQ ID NO: 39 - protein, 17 aa, Artificial Sequence
  4F12 Lv FR2
VYWYQQLPGTAPKLLIY

SEQ ID NO: 40 - protein, 36 aa, Artificial Sequence
  1A03 & 3H10 Lv FR3
NRPSGVPDRFSGSKSGTSASLAISGLRSEDEADYYC

SEQ ID NO: 41 - protein, 36 aa, Artificial Sequence
  4F12 Lv FR3
KRPSGVPDRFSGSKSGTSASLAISGLRSEDEADYYC

SEQ ID NO: 42 - protein, 10 aa, Artificial Sequence
  1A03, 3H10 & 4F12 Lv FR4
FGGGTKLTVL